European Patent Application EP 4 434 579 A1, published September 25, 2024. Title: OBESTATIN FOR USE AS ANTINEOPLASTIC AGENT IN THE TREATMENT OF PANCREATIC CANCER. Applicant: SERVIZO GALEGO DE SAÚDE. The sequence listing filed with the application follows.

SEQUENCE LISTING (18 sequences)

SEQ ID NO: 1 - protein, 23 aa, Homo sapiens
FNAPFDVGIKLSGVQYQQHSQAL

SEQ ID NO: 2 - protein, 23 aa, Equus caballus
FNAPFDVGIKLSGAQYHQHSQAL

SEQ ID NO: 3 - protein, 23 aa, Ailuropoda melanoleuca
FNAPFDVGIKLSGAQYQEHGQAL

SEQ ID NO: 4 - protein, 23 aa, Mesocricetus auratus
FNAPFDVGIKLSGAQYQQHGRAL

SEQ ID NO: 5 - protein, 23 aa, Canis lupus
FNAPFDVGIKLSGPQYHQHGQAL

SEQ ID NO: 6 - protein, 23 aa, Felis catus
FNAPFDVGIKLSGAQYHQHGQAL

SEQ ID NO: 7 - protein, 23 aa, Odocoileus virginianus
FNAPFDIGIKLSGAQSLQHGQTL

SEQ ID NO: 8 - protein, 23 aa, Sus scrofa
FNAPCDVGIKLSGAQSDQHGQPL

SEQ ID NO: 9 - protein, 23 aa, Capra hircus
FNAPFNIGIKLSGAQSLQHGQTL

SEQ ID NO: 10 - protein, 13 aa, Homo sapiens
LSGVQYQQHSQAL

SEQ ID NO: 11 - protein, 13 aa, Equus caballus
LSGAQYHQHSQAL

SEQ ID NO: 12 - protein, 13 aa, Ailuropoda melanoleuca
LSGAQYQEHGQAL

SEQ ID NO: 13 - protein, 13 aa, Mesocricetus auratus
LSGAQYQQHGRAL

SEQ ID NO: 14 - protein, 13 aa, Canis lupus
LSGPQYHQHGQAL

SEQ ID NO: 15 - protein, 13 aa, Felis catus
LSGAQYHQHGQAL

SEQ ID NO: 16 - protein, 13 aa, Odocoileus virginianus
LSGAQSLQHGQTL

SEQ ID NO: 17 - protein, 13 aa, Sus scrofa
LSGAQSDQHGQPL

SEQ ID NO: 18 - protein, 13 aa, Capra hircus
LSGAQSLQHGQTL